European Patent Application EP 4 361 172 A2, published May 1, 2024. Title: Konstrukt do wektora ekspresyjnego do ekspresji rekombinowanej µ-konotoksyny TIIIA lub TIIIAlaMut, zawierający go wektor ekspresyjny, wyizolowana komórka E. coli zawierająca wspomniany wektor ekspresyjny oraz sposób wytwarzania µ-konotoksyny TIIIA lub TIIIAlaMut w E. coli z wektorem ekspresyjnym zawierającym wspomniany konstrukt. Applicant: SCIENCE4BEAUTY SP. Z O.O. The sequence listing filed with the application follows.

SEQUENCE LISTING (7 sequences)

SEQ ID NO: 1 - DNA, 423 bp, unidentified
  source 1..423: mol_type = unassigned DNA
atgcatcaccatcatcaccattctggttcttctgacaaaatcatccacctgaccgacgactctttcgacaccgacgttctgaaagctgacggtgctatcctggttgacttctgggctgaatggtgcggtccgtgcaaaaagatcgctccgatcctggacgaaatcgctgacgaataccagggtaaactgaccgttgctaaactgaacatcgaccagaacccgggtaccgctccgaaatacggtatccgtggtatcccgaccctgctgctgttcaaaaacggtgaagttgctgcaaccaaagttggtgcactgtctaaaggtcagctgaaagaattcctggacgctaacctggctatgcgtcatggctgctgcaaaggcccgaaaggctgcagcagccgtgaatgccgtccgcagcattgctgc

SEQ ID NO: 2 - protein, 141 aa, unidentified
MHHHHHHSGSSDKIIHLTDDSFDTDVLKADGAILVDFWAEWCGPCKKIAPILDEIADEYQGKLTVAKLNIDQNPGTAPKYGIRGIPTLLLFKNGEVAATKVGALSKGQLKEFLDANLAMRHGCCKGPKGCSSRECRPQHCC

SEQ ID NO: 3 - protein, 22 aa, synthetic construct
RHGCCKGPKGCSSRECRPQHCC

SEQ ID NO: 4 - DNA, 423 bp, unidentified
  source 1..423: mol_type = unassigned DNA
atgcatcaccatcatcaccattctggttcttctgacaaaatcatccacctgaccgacgactctttcgacaccgacgttctgaaagctgacggtgctatcctggttgacttctgggctgaatggtgcggtccgtgcaaaaagatcgctccgatcctggacgaaatcgctgacgaataccagggtaaactgaccgttgctaaactgaacatcgaccagaacccgggtaccgctccgaaatacggtatccgtggtatcccgaccctgctgctgttcaaaaacggtgaagttgctgcaaccaaagttggtgcactgtctaaaggtcagctgaaagaattcctggacgctaacctggctatgcgtcatggctgctgcaaaggcccgaaaggctgcagcagccgtgcttgccgtccgcagcattgctgc

SEQ ID NO: 5 - protein, 141 aa, unidentified
MHHHHHHSGSSDKIIHLTDDSFDTDVLKADGAILVDFWAEWCGPCKKIAPILDEIADEYQGKLTVAKLNIDQNPGTAPKYGIRGIPTLLLFKNGEVAATKVGALSKGQLKEFLDANLAMRHGCCKGPKGCSSRACRPQHCC

SEQ ID NO: 6 - DNA, 3869 bp, unidentified
  source 1..3869: mol_type = unassigned DNA
ttctcatgtttgacagcttatcatcgataagctttaatgcggtagtttatcacagttaaattgctaacgcagtcaggcaccgtgtatgaaatctaacaatgcgctcatcgtcatcctcggcaccgtcaccctggatgctgtaggcataggcttggttatgccggtactgccgggcctcttgcgggatatcgtccattccgacagcatcgccagtcactatggcgtgctgctagcgctatatgcgttgatgcaatttctatgcgcacccgttctcggagcactgtccgaccgctttggccgccgcccagtcctgctcgcttcgctacttggagccactatcgactacgcgatcatggcgaccacacccgtcctgtggatcctctacgccggacgcatcgtggccggcatcaccggcgccacaggtgcggttgctggcgcctatatcgccgacatcaccgatggggaagatcgggctcgccacttcgggctcatgagcgcttgtttcggcgtgggtatggtggcaggccccgtggccgggggactgttgggcgccatctccttgcatgcaccattccttgcggcggcggtgctcaacggcctcaacctactactgggctgcttcctaatgcaggagtcgcataagggagagcgtcgaccgatgcccttgagagccttcaacccagtcagctccttccggtgggcgcggggcatgactatcgtcgccgcacttatgactgtcttctttatcatgcaactcgtaggacaggtgccggcagcgctctgggtcattttcggcgaggaccgctttcgctggagcgcgacgatgatcggcctgtcgcttgcggtattcggaatcttgcacgccctcgctcaagccttcgtcactggtcccgccaccaaacgtttcggcgagaagcaggccattatcgccggcatggcggccgacgcgctgggctacgtcttgctggcgttcgcgacgcgaggctggatggccttccccattatgattcttctcgcttccggcggcatcgggatgcccgcgttgcaggccatgctgtccaggcaggtagatgacgaccatcagggacagcttcaaggatcgctcgcggctcttaccagcctaacttcgatcattggaccgctgatcgtcacggcgatttatgccgcctcggcgagcacatggaacgggttggcatggattgtaggcgccgccctataccttgtctgcctccccgcgttgcgtcgcggtgcatggagccgggccacctcgacctgaatggaagccggcggcacctcgctaacggattcaccactccaagaattggagccaatcaattcttgcggagaactgtgaatgcgcaaaccaacccttggcagaacatatccatcgcgtccgccatctccagcagccgcacgcggcgcatctcgggcagcgttgggtcctggccacgggtgcgcatgatcgtgctcctgtcgttgagtaatacggttatccacagaatcaggggataacgcaggaaagaacatgtgagcaaaaggccagcaaaaggccaggaaccgtaaaaaggccgcgttgctggcgtttttccataggctccgcccccctgacgagcatcacaaaaatcgacgctcaagtcagaggtggcgaaacccgacaggactataaagataccaggcgtttccccctggaagctccctcgtgcgctctcctgttccgaccctgccgcttaccggatacctgtccgcctttctcccttcgggaagcgtggcgctttctcatagctcacgctgtaggtatctcagttcggtgtaggtcgttcgctccaagctgggctgtgtgcacgaaccccccgttcagcccgaccgctgcgccttatccggtaactatcgtcttgagtccaacccggtaagacacgacttatcgccactggcagcagccactggtaacaggattagcagagcgaggtatgtaggcggtgctacagagttcttgaagtggtggcctaactacggctacactagaaggacagtatttggtatctgcgctctgctgaagccagttaccttcggaaaaagagttggtagctcttgatccggcaaacaaaccaccgctggtagcggtggtttttttgtttgcaagcagcagattacgcgcagaaaaaaaggatctcaagaagatcctttgatcttttctacggggtctgacgctcagtggaacgaaaactcacgttaacgatcgatttttggtgataatgtcccaaatatgtcccactctgaaattatggaggatataaagaaggcgtaactgattgaattgtaatggcgcgccctgcaggattcgaacctgcggcccacgacttagaaggtcgttgctctatccaactgagctaagggcgcgttgataccgcaatgcggtgtaatcgcgtgaattatacggtcaacccttgctgagtcaatggcttttgatctgggagctcgggaccgttggcgatgtgcggtttgctacattcacagatgttcttcgccacttccagcagcaggtcatcaggggtgatttcaggatcgtagataaaggtcaggttcggtgaaacctgcttcaactctgcatctgcacgtaagatcgcgcgggtaatgggcgaatcagacgggccgatattggcgtgcataaaggcgtctggcagggttctgtcgaggtaacgccagaaacgttttattcgaacatcgatctcgtcttgtgttagaattaattctaacatacggttgcaacaacgcatccagttgccccaggtagaccggcatcgatgtgaccgacggtacgtggtggtaaagaatggtcagcagagagagtgcgtcatcaagatctttcgcgccttccagctccagccattcggaaccgttcgccagaaaacgggcgtaatcgggtaagacatagcgcggtttgtacggcgcatgaccttcaaacatatcgcagattacaccttcatccagcgcgcggcgggcttcggcaggaagctgtgggtaaggcagattgttttctgcttccagtgccagaaaatggcgcttctgctccgggctaagcactgggctggtgacaatttgctggcaacgttgttgcagtgcattttcatgagaagtgggcatcttcttttccttttatgccgaaggtgatgcgccattgtaagaagtttcgtgatgttcactttgatcctgatgcgtttgccaccactgacgcattcatttgaaagtgaattatttgaaccagatcgcattacagtgatgcaaacttgtaagtagatttccttaattgtgatgtgtatcgaagtgtgttgcggagtagatgttagaatactaacaaactcgcaaggtgaattttattggcgacaagcctaggtttgtttaactttaaggagaaatcatatgcatcaccatcatcaccattctggttcttctgacaaaatcatccacctgaccgacgactctttcgacaccgacgttctgaaagctgacggtgctatcctggttgacttctgggctgaatggtgcggtccgtgcaaaaagatcgctccgatcctggacgaaatcgctgacgaataccagggtaaactgaccgttgctaaactgaacatcgaccagaacccgggtaccgctccgaaatacggtatccgtggtatcccgaccctgctgctgttcaaaaacggtgaagttgctgcaaccaaagttggtgcactgtctaaaggtcagctgaaagaattcctggacgctaacctggctatgcgtcatggctgctgcaaaggcccgaaaggctgcagcagccgtgaatgccgtccgcagcattgctgctaatctagactcgagttcgtcttcaagaa

SEQ ID NO: 7 - DNA, 4462 bp, unidentified
  source 1..4462: mol_type = unassigned DNA
ggaccgttggcgatgtgcggtttgctacattcacagatgttcttcgccacttccagcagcaggtcatcaggggtgatttcaggatcgtagataaaggtcaggttcggtgaaacctgcttcaactctgcatctgcacgtaagatcgcgcgggtaatgggcgaatcagacgggccgatattggcgtgcataaaggcgtctggcagggttctgtcgaggtaacgccagaaacgttttattcgaacatcgatctcgtcttgtgttagaattaattctaacatacggttgcaacaacgcatccagttgccccaggtagaccggcatcgatgtgaccgacggtacgtggtggtaaagaatggtcagcagagagagtgcgtcatcaagatctttcgcgccttccagctccagccattcggaaccgttcgccagaaaacgggcgtaatcgggtaagacatagcgcggtttgtacggcgcatgaccttcaaacatatcgcagattacaccttcatccagcgcgcggcgggcttcggcaggaagctgtgggtaaggcagattgttttctgcttccagtgccagaaaatggcgcttctgctccgggctaagcactgggctggtgacaatttgctggcaacgttgttgcagtgcattttcatgagaagtgggcatcttcttttccttttatgccgaaggtgatgcgccattgtaagaagtttcgtgatgttcactttgatcctgatgcgtttgccaccactgacgcattcatttgaaagtgaattatttgaaccagatcgcattacagtgatgcaaacttgtaagtagatttccttaattgtgatgtgtatcgaagtgtgttgcggagtagatgttagaatactaacaaactcgcaaggtgaattttattggcgacaagcctaggtttgtttaactttaaggagaaatcatatgcatcaccatcatcaccattctggttcttctgacaaaatcatccacctgaccgacgactctttcgacaccgacgttctgaaagctgacggtgctatcctggttgacttctgggctgaatggtgcggtccgtgcaaaaagatcgctccgatcctggacgaaatcgctgacgaataccagggtaaactgaccgttgctaaactgaacatcgaccagaacccgggtaccgctccgaaatacggtatccgtggtatcccgaccctgctgctgttcaaaaacggtgaagttgctgcaaccaaagttggtgcactgtctaaaggtcagctgaaagaattcctggacgctaacctggctatgcgtcatggctgctgcaaaggcccgaaaggctgcagcagccgtgaatgccgtccgcagcattgctgctaatctagagtcgacctgcaggcatgcaagcttagcccgcttaatgagcgggcttttttttctcgaggacgtctaagaaaccattattatcatgacattaacctataaaaataggcgtatcacgaggccctttcgtcttcaagaattctcatgtttgacagcttatcatcgataagctttaatgcggtagtttatcacagttaaattgctaacgcagtcaggcaccgtgtatgaaatctaacaatgcgctcatcgtcatcctcggcaccgtcaccctggatgctgtaggcataggcttggttatgccggtactgccgggcctcttgcgggatatcgtccattccgacagcatcgccagtcactatggcgtgctgctagcgctatatgcgttgatgcaatttctatgcgcacccgttctcggagcactgtccgaccgctttggccgccgcccagtcctgctcgcttcgctacttggagccactatcgactacgcgatcatggcgaccacacccgtcctgtggatcctctacgccggacgcatcgtggccggcatcaccggcgccacaggtgcggttgctggcgcctatatcgccgacatcaccgatggggaagatcgggctcgccacttcgggctcatgagcgcttgtttcggcgtgggtatggtggcaggccccgtggccgggggactgttgggcgccatctccttgcatgcaccattccttgcggcggcggtgctcaacggcctcaacctactactgggctgcttcctaatgcaggagtcgcataagggagagcgtcgaccgatgcccttgagagccttcaacccagtcagctccttccggtgggcgcggggcatgactatcgtcgccgcacttatgactgtcttctttatcatgcaactcgtaggacaggtgccggcagcgctctgggtcattttcggcgaggaccgctttcgctggagcgcgacgatgatcggcctgtcgcttgcggtattcggaatcttgcacgccctcgctcaagccttcgtcactggtcccgccaccaaacgtttcggcgagaagcaggccattatcgccggcatggcggccgacgcgctgggctacgtcttgctggcgttcgcgacgcgaggctggatggccttccccattatgattcttctcgcttccggcggcatcgggatgcccgcgttgcaggccatgctgtccaggcaggtagatgacgaccatcagggacagcttcaaggatcgctcgcggctcttaccagcctaacttcgatcattggaccgctgatcgtcacggcgatttatgccgcctcggcgagcacatggaacgggttggcatggattgtaggcgccgccctataccttgtctgcctccccgcgttgcgtcgcggtgcatggagccgggccacctcgacctgaatggaagccggcggcacctcgctaacggattcaccactccaagaattggagccaatcaattcttgcggagaactgtgaatgcgcaaaccaacccttggcagaacatatccatcgcgtccgccatctccagcagccgcacgcggcgcatctcgggcagcgttgggtcctggactcaccagtcacagaaaagcatcttacggatggcatgacagtaagagaattatgcagtgctgccataaccatgagtgataacactgcggccaacttacttctgacaacgatcggaggaccgaaggagctaaccgcttttttgcacaacatgggggatcatgtaactcgccttgatcgttgggaaccggagctgaatgaagccataccaaacgacgagcgtgacaccacgatgcctgcagcaatggcaacaacgttgcgcaaactattaactggcgaactacttactctagcttcccggcaacaattaatagactggatggaggcggataaagttgcaggaccacttctgcgctcggcccttccggctggctggtttattgctgataaatctggagccggtgagcgtgggtctcgcggtatcattgcagcactggggccagatggtaagccctcccgtatcgtagttatctacacgacggggagtcaggcaactatggatgaacgaaatagacagatcgctgagataggtgcctcactgattaagcattggtaactgtcagaccaagtttactcatatatactttagattgatttaaaacttcatttttaatttaaaaggatctaggtgaagatcctttttgataatctcatgaccaaaatcccttaacgtgagttttcgttccactgagcgtcagaccccgtagaaaagatcaaaggatcttcttgagatcaaaggatcttcttgagatcctttttttctgcgcgtaatctgctgcttgcaaacaaaaaaaccaccgctaccagcggtggtttgtttgccggatcaagagctaccaactctttttccgaaggtaactggcttcagcagagcgcagataccaaatactgtccttctagtgtagccgtagttaggccaccacttcaagaactctgtagcaccgcctacatacctcgctctgctaatcctgttaccagtggctgctgccagtggcgataagtcgtgtcttaccgggttggactcaagacgatagttaccggataaggcgcagcggtcgggctgaacggggggttcgtgcacacagcccagcttggagcgaacgacctacaccgaactgagatacctacagcgtgagctatgagaaagcgccacgcttcccgaagggagaaaggcggacaggtatccggtaagcggcagggtcggaacaggagagcgcacgagggagcttccagggggaaacgcctggtatctttatagtcctgtcgggtttcgccacctctgacttgagcgtcgatttttgtgatgctcgtcaggggggcggagcctatggaaaaacgccagcaacgcggcctttttacggttcctggccttttgctggccttttgctcacatgttctttcctgcgttatcccctgattctgtggataaccgtattaccgcctttgagtgagctgataccgctcgccgcagccgaacgaccgagcgcagcgagtcagtgaggatcgatccg